European Patent Application EP 4 458 851 A1, published November 6, 2024. Title: 抗GPRC5D抗体及其应用. Applicant: 康源博创生物科技（北京）有限公司. The sequence listing filed with the application follows.

SEQUENCE LISTING (54 sequences)

SEQ ID NO: 1 - protein, 118 aa, synthetic construct
  REGION 1..118: note = VH
QVQLVQSGAEVKKPGASVKVSCKASGYSFTGYTMNWVRQAPGQGLEWMGLINPYNSDTNYAQKLQGRVTMTTDTSTSTAYMELRSLRSDDTAVYYCARVALRVALDYWGQGTLVTVSS

SEQ ID NO: 2 - protein, 109 aa, synthetic construct
  REGION 1..109: note = VL
QTVVTQEPSLTVSPGGTVTLTCRSSTGAVTTSNYANWVQQKPGQAPRGLIGGTNKRAPGTPARFSGSLLGGKAALTLSGVQPEDEAEYYCALWYSNLWVFGGGTKLTVL

SEQ ID NO: 3 - protein, 107 aa, synthetic construct
  REGION 1..107: note = VL
DIQMTQSPSSLSASVGDRVTITCKASQNVATHVGWYQQKPGKAPKRLIYSASYRYSGVPSRFSGSGSGTEFTLTISNLQPEDFATYYCQQYNRYPYTFGQGTKLEIK

SEQ ID NO: 4 - protein, 125 aa, synthetic construct
  REGION 1..125: note = VH
EVQLVESGGGLVQPGGSLRLSCAASGFTFNTYAMNWVRQAPGKGLEWVARIRSKYNNYATYYAASVKGRFTISRDDSKNSLYLQMNSLKTEDTAVYYCARHGNFGNSYVSWFAYWGQGTLVTVSS

SEQ ID NO: 5 - protein, 123 aa, synthetic construct
  REGION 1..123: note = VH
QVQLKESGPGLVKPSQSLSLTCTVTGYSITSDYAWNWIRQFPGNKLEWMGYISYSGSATYNPSLKSRISITRDTSKNQFFLQLNSMTTEDTATYYCARGGIAGRGRWGAMDYWGQGTSVTVSS

SEQ ID NO: 6 - protein, 107 aa, synthetic construct
  REGION 1..107: note = VL
DIVMTQAQKFMSTSVGDRVSVTCKASQNVGTNVAWYQNKPGQSPKALIYSASYRDSGVPDRFTGRGSGTDFTLTISNVQSEDLAEYFCQQYKSYPLTFGAGTKLELK

SEQ ID NO: 7 - protein, 118 aa, synthetic construct
  REGION 1..118: note = VH
QVQLKQSGAELAGPGASVKMSCKASGYTFTSYTIQWIKQRPGQGLEWIGYIIPSSGYTNYNQKFKDKATLTADKSSNTAYMQLSSLTSEDSAVYYCANNYGNWGFTYWGQGTLVTVSA

SEQ ID NO: 8 - protein, 107 aa, synthetic construct
  REGION 1..107: note = VL
DILMTQSQKFMSTSVRDRVSISCKASQNVGSAVTWYQQKPGQSPRLLIYSASNRYTGVPDRFTGSGSGTDFTLTISNVQSEDLADYFCQQYSNYPLTFGGGTKLEIK

SEQ ID NO: 9 - protein, 118 aa, synthetic construct
  REGION 1..118: note = VH
QVQLKESGPELVKPGASVKISCKASGYTFPYYVMHWVKQKPGQGLEWIGYINPYNDGTKYNEKFKGKAALTSDKSSSTAYMDLSSLTSEDSAVYYCARGGVRRYFDYWGQGTTLTVSS

SEQ ID NO: 10 - protein, 107 aa, synthetic construct
  REGION 1..107: note = VL
DIQMTQTPSSLSASLGERVSLTCRASQDIGSNLNWLQQEPDGTIKRLIYATSSLDSGVPKRFSGSRSGSDYSLTISSLESEDFVDYYCLQYATFPYTFGGGTKLEIK

SEQ ID NO: 11 - protein, 118 aa, synthetic construct
  REGION 1..118: note = VH
QVQLKESGPELVKPGASVKISCKASGYTFPYYVIHWVKQKPGQGLEWIGYINPYNDGTKYNEKFKGKAALTSDKSSSTAYMELSSLTSEDSAVYYCARGGVRRYFDYWGQGTTLTVSS

SEQ ID NO: 12 - protein, 107 aa, synthetic construct
  REGION 1..107: note = VL
QIVLTQSPSSLSASLGERVSLTCRASQDIGSNLNWLQQEPDGTIKRLISATSSLDSGVPKRFSGSRSGSDYSLTISSLESEDFVDYFCLQYATFPYTFGGGTKLEIK

SEQ ID NO: 13 - protein, 123 aa, synthetic construct
  REGION 1..123: note = VH
QVQLQESGPGLVKPSETLSLTCTVSGYSITSDYAWNWIRQPPGKGLEWMGYISYSGSATYSPSLKSRITISRDTSKNQFSLKLSSVTAADTAVYYCARGGIAGRGRWGAMDYWGQGTTVTVSS

SEQ ID NO: 14 - protein, 107 aa, synthetic construct
  REGION 1..107: note = VL
DIQMTQSPSSLSASVGDRVTITCKASQNVGTNVAWYQQKPGQSPKALIYSASYRDSGVPDRFSGSGSGTDFTLTISSLQPEDFATYYCQQYKSYPLTFGQGTRLEIK

SEQ ID NO: 15 - protein, 118 aa, synthetic construct
  REGION 1..118: note = VH
QVQLVQSGAEVKKPGASVKVSCKASGYTFTSYTIQWIKQAPGQGLEWIGYIIPSSGYTNYNQKFKDKATLTADKSSNTAYMELSSLTSEDTAVYYCANNYGNWGFTYWGQGTTVTVSS

SEQ ID NO: 16 - protein, 107 aa, synthetic construct
  REGION 1..107: note = VL
DIQMTQSPSTLSASVGDRVTITCKASQNVGSAVTWYQQKPGKAPRLLIYSASNRYTGVPDRFSGSGSGTEFTLTISSLQPDDFATYFCQQYSNYPLTFGQGTRLEIK

SEQ ID NO: 17 - protein, 118 aa, synthetic construct
  REGION 1..118: note = VH
QVQLVQSGAEVKKPGASVKVSCKASGYTFPYYVMHWVRQAPGQGLEWIGYINPYNDGTKYNEKFKGRATLTSDKSTSTAYMELSSLRSEDTAVYYCARGGVRRYFDYWGQGTTVTVSS

SEQ ID NO: 18 - protein, 107 aa, synthetic construct
  REGION 1..107: note = VL
DIQMTQSPSTLSASVGDRVTITCRASQDIGSNLNWLQQKPGGTIKRLIYATSSLDSGVPSRFSGSRSGSEYTLTISSLQPDDFATYYCLQYATFPYTFGQGTRLEIK

SEQ ID NO: 19 - protein, 118 aa, synthetic construct
  REGION 1..118: note = VH
QVQLVQSGAEVKKPGASVKVSCKASGYTFPYYVIHWVRQAPGQGLEWIGYINPYNAGTKYNEKFKGRATLTSDKSTSTAYMELSSLRSEDTAVYYCARGGVRRYFDYWGQGTTVTVSS

SEQ ID NO: 20 - protein, 107 aa, synthetic construct
  REGION 1..107: note = VL
DIQLTQSPSTLSASVGDRVTITCRASQDIGSNLNWLQQKPGGTIKRLISATSSLDSGVPSRFSGSRSGSEYTLTISSLQPDDFATYYCLQYATFPYTFGQGTRLEIK

SEQ ID NO: 21 - protein, 125 aa, synthetic construct
  REGION 1..125: note = VH
QVQLVESGGGLVKPGGSLRLSCAASGFTFSTYAMNWVRQAPGKGLEWVGRIRSKYNNYATYYADSVKDRFTISRDDAKNSLYLQMNSLRAEDTAVYYCARHGNFGNSYVSYFAYWGQGTTVTVSS

SEQ ID NO: 22 - protein, 110 aa, synthetic construct
  REGION 1..110: note = VL
DIQMTQSPSSLSASVGDRVTITCRSSTGAVTTSNYANWVQQKPGKAPKALIGGTNKRAPGVPSRFSGSLSGDDATLTISSLQPEDFATYYCALWYSNLWVFGQGTRLEIK

SEQ ID NO: 23 - protein, 330 aa, synthetic construct [sequence omitted]

SEQ ID NO: 24 - protein, 107 aa, synthetic construct [sequence omitted]

SEQ ID NO: 25 - protein, 329 aa, synthetic construct
  REGION 1..329: note = CH1-CH2-CH3
ASTKGPSVFPLAPSSKSTSGGTAALGCLVKDYFPEPVTVSWNSGALTSGVHTFPAVLQSSGLYSLSSVVTVPSSSLGTQTYICNVNHKPSNTKVDKRVEPKSCDKTHTCPPCPAPPAAGPSVFLFPPKPKDTLMISRTPEVTCVVVDVSHEDPEVKFNWYVDGVEVHNAKTKPREEQYNSTYRVVSVLTVLHQDWLNGKEYKCKVSNKALAAPIEKTISKAKGQPREPQVYTLPPCREEMTKNQVSLWCLVKGFYPSDIAVEWESNGQPENNYKTTPPVLDSDGSFLLYSKLTVDKSRWQQGNVFSCSVMHEALHNHYTQKSLSLSPGK

SEQ ID NO: 26 - protein, 331 aa, synthetic construct
  REGION 1..331: note = CH1-CH2-CH3
SSASTKGPSVFPLAPSSKSTSGGTAALGCLVEDYFPEPVTVSWNSGALTSGVHTFPAVLQSSGLYSLSSVVTVPSSSLGTQTYICNVNHKPSNTKVDDRVEPKSCDKTHTCPPCPAPPAAGPSVFLFPPKPKDTLMISRTPEVTCVVVDVSHEDPEVKFNWYVDGVEVHNAKTKPREEQYNSTYRVVSVLTVLHQDWLNGKEYKCKVSNKALAAPIEKTISKAKGQPREPQVCTLPPSREEMTKNQVSLSCAVKGFYPSDIAVEWESNGQPENNYKTTPPVLDSDGSFFLVSRLTVDKSRWQQGNVFSCSVMHEALHNHYTQKSLSLSPGK

SEQ ID NO: 27 - protein, 106 aa, synthetic construct
  REGION 1..106: note = CL
GQPKAAPSVTLFPPSSEELQANKATLVCLISDFYPGAVTVAWKADSSPVKAGVETTTPSKQSNNKYAASSYLSLTPEQWKSHRSYSCQVTHEGSTVEKTVAPTECS

SEQ ID NO: 28 - protein, 6 aa, synthetic construct
  REGION 1..6: note = HCDR-1
SDYAWN

SEQ ID NO: 29 - protein, 16 aa, synthetic construct
  REGION 1..16: note = HCDR-2
YISYSGSATYNPSLKS

SEQ ID NO: 30 - protein, 14 aa, synthetic construct
  REGION 1..14: note = HCDR-3
GGIAGRGRWGAMDY

SEQ ID NO: 31 - protein, 11 aa, synthetic construct
  REGION 1..11: note = LCDR-1
KASQNVGTNVA

SEQ ID NO: 32 - protein, 7 aa, synthetic construct
  REGION 1..7: note = LCDR-2
SASYRDS

SEQ ID NO: 33 - protein, 9 aa, synthetic construct
  REGION 1..9: note = LCDR-3
QQYKSYPLT

SEQ ID NO: 34 - protein, 16 aa, synthetic construct
  REGION 1..16: note = HCDR-2
YISYSGSATYSPSLKS

SEQ ID NO: 35 - protein, 5 aa, synthetic construct
  REGION 1..5: note = HCDR-1
SYTIQ

SEQ ID NO: 36 - protein, 17 aa, synthetic construct
  REGION 1..17: note = HCDR-2
YIIPSSGYTNYNQKFKD

SEQ ID NO: 37 - protein, 9 aa, synthetic construct
  REGION 1..9: note = HCDR-3
NYGNWGFTY

SEQ ID NO: 38 - protein, 11 aa, synthetic construct
  REGION 1..11: note = LCDR-1
KASQNVGSAVT

SEQ ID NO: 39 - protein, 7 aa, synthetic construct
  REGION 1..7: note = LCDR-2
SASNRYT

SEQ ID NO: 40 - protein, 9 aa, synthetic construct
  REGION 1..9: note = LCDR-3
QQYSNYPLT

SEQ ID NO: 41 - protein, 5 aa, synthetic construct
  REGION 1..5: note = HCDR-1
YYVMH

SEQ ID NO: 42 - protein, 17 aa, synthetic construct
  REGION 1..17: note = HCDR-2
YINPYNDGTKYNEKFKG

SEQ ID NO: 43 - protein, 9 aa, synthetic construct
  REGION 1..9: note = HCDR-3
GGVRRYFDY

SEQ ID NO: 44 - protein, 11 aa, synthetic construct
  REGION 1..11: note = LCDR-1
RASQDIGSNLN

SEQ ID NO: 45 - protein, 7 aa, synthetic construct
  REGION 1..7: note = LCDR-2
ATSSLDS

SEQ ID NO: 46 - protein, 9 aa, synthetic construct
  REGION 1..9: note = LCDR-3
LQYATFPYT

SEQ ID NO: 47 - protein, 5 aa, synthetic construct
  REGION 1..5: note = HCDR-1
YYVIH

SEQ ID NO: 48 - protein, 17 aa, synthetic construct
  REGION 1..17: note = HCDR-2
YINPYNAGTKYNEKFKG

SEQ ID NO: 49 - protein, 5 aa, synthetic construct
  REGION 1..5: note = HCDR-1
TYAMN

SEQ ID NO: 50 - protein, 19 aa, synthetic construct
  REGION 1..19: note = HCDR-2
RIRSKYNNYATYYADSVKD

SEQ ID NO: 51 - protein, 14 aa, synthetic construct
  REGION 1..14: note = HCDR-3
HGNFGNSYVSYFAY

SEQ ID NO: 52 - protein, 14 aa, synthetic construct
  REGION 1..14: note = LCDR-1
RSSTGAVTTSNYAN

SEQ ID NO: 53 - protein, 7 aa, synthetic construct
  REGION 1..7: note = LCDR-2
GTNKRAP

SEQ ID NO: 54 - protein, 9 aa, synthetic construct
  REGION 1..9: note = LCDR-3
ALWYSNLWV